European Patent Application EP 4 501 356 A1, published February 5, 2025. Title: Removal of senescent cells by ammonia-lowering components. Applicant: 株式会社ファンタジーン. Application JP. The sequence listing filed with the application follows.

SEQUENCE LISTING (4 sequences)

SEQ ID NO: 1 - DNA, 20 bp, synthetic construct
  misc_feature 1..20: note = Forward primer for p16 gene
  source 1..20: mol_type = other DNA
cgtaccccgattcaggtgat

SEQ ID NO: 2 - DNA, 22 bp, synthetic construct
  misc_feature 1..22: note = Reverse primer for p16 gene
  source 1..22: mol_type = other DNA
ttgagcagaagagctgctacgt

SEQ ID NO: 3 - DNA, 19 bp, synthetic construct
  misc_feature 1..19: note = Forward primer for p21 gene
  source 1..19: mol_type = other DNA
cctggtgatgtccgacctg

SEQ ID NO: 4 - DNA, 19 bp, synthetic construct
  misc_feature 1..19: note = Reverse primer for p21 gene
  source 1..19: mol_type = other DNA
ccatgagcgcatcgcaatc